European Patent Application EP 4 464 722 A1, published November 20, 2024. Title: 一种抗体及其用途. Applicant: 南京维立志博生物科技有限公司. Application WO. The sequence listing filed with the application follows.

SEQUENCE LISTING (128 sequences)

SEQ ID NO: 1 - protein, 455 aa, artificial sequence
EVQLVESGGGLVQPGGSLKLSCAASGFTFSTYAMNWVRQAPGKGLEWVGRIRSKYNNYATYYADSVKDRFTISRDDSKNTLYLQMNSLKTEDTAVYYCTRHGNFGNSYVSWFAYWGQGTTVTVSSASTKGPSVFPLAPSSKSTSGGTAALGCLVKDYFPEPVTVSWNSGALTSGVHTFPAVLQSSGLYSLSSVVTVPSSSLGTQTYICNVNHKPSNTKVDKKVEPKSCDKTHTCPPCPAPEAAGGPSVFLFPPKPKDTLMISRTPEVTCVVVAVSHEDPEVKFNWYVDGVEVHNAKTKPREEQYNSTYRVVSVLTVLHQDWLNGKEYKCKVSNKALAAPIEKTISKAKGQPREPQVYTLPPSRDELTKNQVSLTCLVKGFYPSDIAVEWESNGQPENNYKTTPPVLDSDGSFFLYSKLTVDKSRWQQGNVFSCSVMHEALHNHYTQKSLSLSPGK

SEQ ID NO: 2 - protein, 214 aa, artificial sequence
QAVVTQEPSLTVSPGGTVTLTCRSSTGAVTTSNYANWVQQKPGQAPRGLIGGTNKRAPGVPARFSGSLLGGKAALTLSGAQPEDEAEYFCALWYSNLWVFGGGTKLTVLGQPKAAPSVTLFPPSSEELQANKATLVCLISDFYPGAVTVAWKADSSPVKAGVETTTPSKQSNNKYAASSYLSLTPEQWKSHRSYSCQVTHEGSTVEKTVAPTEC

SEQ ID NO: 3 - protein, 125 aa, artificial sequence
EVQLVESGGGLVQPGGSLKLSCAASGFTFSTYAMNWVRQAPGKGLEWVGRIRSKYNNYATYYADSVKDRFTISRDDSKNTLYLQMNSLKTEDTAVYYCTRHGNFGNSYVSWFAYWGQGTTVTVSS

SEQ ID NO: 4 - protein, 109 aa, artificial sequence
QAVVTQEPSLTVSPGGTVTLTCRSSTGAVTTSNYANWVQQKPGQAPRGLIGGTNKRAPGVPARFSGSLLGGKAALTLSGAQPEDEAEYFCALWYSNLWVFGGGTKLTVL

SEQ ID NO: 5 - protein, 5 aa, artificial sequence
TYAMN

SEQ ID NO: 6 - protein, 19 aa, artificial sequence
RIRSKYNNYATYYADSVKD

SEQ ID NO: 7 - protein, 14 aa, artificial sequence
HGNFGNSYVSWFAY

SEQ ID NO: 8 - protein, 14 aa, artificial sequence
RSSTGAVTTSNYAN

SEQ ID NO: 9 - protein, 7 aa, artificial sequence
GTNKRAP

SEQ ID NO: 10 - protein, 9 aa, artificial sequence
ALWYSNLWV

SEQ ID NO: 11 - protein, 250 aa, artificial sequence
EVQLVESGGGLVQPGGSLKLSCAASGFTFSTYAMNWVRQAPGKGLEWVGRIRSKYNNYATYYADSVKDRFTISRDDSKNTLYLQMNSLKTEDTAVYYCTRHGNFGNSYVSWFAYWGQGTTVTVSSGGGGSGGGGSGGGGSQAVVTQEPSLTVSPGGTVTLTCRSSTGAVTTSNYANWVQQKPGQAPRGLIGGTNKRAPGVPARFSGSLLGGKAALTLSGAQPEDEAEYFCALWYSNLWVFGGGTKLTVLG

SEQ ID NO: 12 - protein, 15 aa, artificial sequence
GGGGSGGGGSGGGGS

SEQ ID NO: 13 - protein, 477 aa, artificial sequence
EVQLVESGGGLVQPGGSLKLSCAASGFTFSTYAMNWVRQAPGKGLEWVGRIRSKYNNYATYYADSVKDRFTISRDDSKNTLYLQMNSLKTEDTAVYYCTRHGNFGNSYVSWFAYWGQGTTVTVSSGGGGSGGGGSGGGGSQAVVTQEPSLTVSPGGTVTLTCRSSTGAVTTSNYANWVQQKPGQAPRGLIGGTNKRAPGVPARFSGSLLGGKAALTLSGAQPEDEAEYFCALWYSNLWVFGGGTKLTVLGDKTHTCPPCPAPEAAGGPSVFLFPPKPKDTLMISRTPEVTCVVVAVSHEDPEVKFNWYVDGVEVHNAKTKPREEQYNSTYRVVSVLTVLHQDWLNGKEYKCKVSNKALAAPIEKTISKAKGQPREPQVYTLPPSRDELTKNQVSLTCLVKGFYPSDIAVEWESNGQPENNYKTTPPVLDSDGSFFLYSKLTVDKSRWQQGNVFSCSVMHEALHNHYTQKSLSLSPGK

SEQ ID NO: 14 - protein, 449 aa, artificial sequence
QVQLVQSGAEVKKPGASVKVSCKASGYTFTTHYMYWVRQAPGQGLEWMGGINPSNGATNFNEKFKTRVTLTVDKSTSTAYMELSSLRSEDTAVYYCTRVGGLSYTMDYWGQGTLVTVSSASTKGPSVFPLAPSSKSTSGGTAALGCLVKDYFPEPVTVSWNSGALTSGVHTFPAVLQSSGLYSLSSVVTVPSSSLGTQTYICNVNHKPSNTKVDKKVEPKSCDKTHTCPPCPAPELLGGPSVFLFPPKPKDTLMISRTPEVTCVVVDVSHEDPEVKFNWYVDGVEVHNAKTKPREEQYNSTYRVVSVLTVLHQDWLNGKEYKCKVSNKALPAPIEKTISKAKGQPREPQVYTLPPSRDELTKNQVSLTCLVKGFYPSDIAVEWESNGQPENNYKTTPPVLDSDGSFFLYSKLTVDKSRWQQGNVFSCSVMHEALHNHYTQKSLSLSPGK

SEQ ID NO: 15 - protein, 220 aa, artificial sequence
DIVMTQSPDSLAVSLGERATINCKSSQSLLYSSNQKNYLAWYQQKPGQPPKLLIYWASTRESGVPDRFSGSGYGTDFTLTISSLQAEDVAVYYCQQYYSYPRTFGGGTKVEIKRTVAAPSVFIFPPSDEQLKSGTASVVCLLNNFYPREAKVQWKVDNALQSGNSQESVTEQDSKDSTYSLSSTLTLSKADYEKHKVYACEVTHQGLSSPVTKSFNRGEC

SEQ ID NO: 16 - protein, 119 aa, artificial sequence
QVQLVQSGAEVKKPGASVKVSCKASGYTFTTHYMYWVRQAPGQGLEWMGGINPSNGATNFNEKFKTRVTLTVDKSTSTAYMELSSLRSEDTAVYYCTRVGGLSYTMDYWGQGTLVTVSS

SEQ ID NO: 17 - protein, 113 aa, artificial sequence
DIVMTQSPDSLAVSLGERATINCKSSQSLLYSSNQKNYLAWYQQKPGQPPKLLIYWASTRESGVPDRFSGSGYGTDFTLTISSLQAEDVAVYYCQQYYSYPRTFGGGTKVEIK

SEQ ID NO: 18 - protein, 220 aa, artificial sequence
DIVMTQSPDSLAVSLGERATINCKSSQSLLYSSNQKNYLAWYQQKPGQPPKLLIYWASTRESGVPDRFSGSGSGTDFTLTISSLQAEDVAVYYCQQYYSYPRTFGGGTKVEIKRTVAAPSVFIFPPSDEQLKSGTASVVCLLNNFYPREAKVQWKVDNALQSGNSQESVTEQDSKDSTYSLSSTLTLSKADYEKHKVYACEVTHQGLSSPVTKSFNRGEC

SEQ ID NO: 19 - protein, 113 aa, artificial sequence
DIVMTQSPDSLAVSLGERATINCKSSQSLLYSSNQKNYLAWYQQKPGQPPKLLIYWASTRESGVPDRFSGSGSGTDFTLTISSLQAEDVAVYYCQQYYSYPRTFGGGTKVEIK

SEQ ID NO: 20 - protein, 220 aa, artificial sequence
DIVMTQSPDSLAVSLGERVTMNCKSSQSLLYSSNQKNYLAWYQQKPGQPPKLLIYWASTRESGVPDRFSGSGYGTDFTLTISSLQAEDVAVYYCQQYYSYPRTFGGGTKLEIKRTVAAPSVFIFPPSDEQLKSGTASVVCLLNNFYPREAKVQWKVDNALQSGNSQESVTEQDSKDSTYSLSSTLTLSKADYEKHKVYACEVTHQGLSSPVTKSFNRGEC

SEQ ID NO: 21 - protein, 113 aa, artificial sequence
DIVMTQSPDSLAVSLGERVTMNCKSSQSLLYSSNQKNYLAWYQQKPGQPPKLLIYWASTRESGVPDRFSGSGYGTDFTLTISSLQAEDVAVYYCQQYYSYPRTFGGGTKLEIK

SEQ ID NO: 22 - protein, 449 aa, artificial sequence
QVQLVQSGAEVKKPGASVKVSCKASGYTFTTHYMYWVRQAPGQGLEWIGGINPSNGATNFNEKFKTKATLTVDKSTSTAYMELSSLRSEDTAVYYCTRVGGLSYTMDYWGQGTLVTVSSASTKGPSVFPLAPSSKSTSGGTAALGCLVKDYFPEPVTVSWNSGALTSGVHTFPAVLQSSGLYSLSSVVTVPSSSLGTQTYICNVNHKPSNTKVDKKVEPKSCDKTHTCPPCPAPELLGGPSVFLFPPKPKDTLMISRTPEVTCVVVDVSHEDPEVKFNWYVDGVEVHNAKTKPREEQYNSTYRVVSVLTVLHQDWLNGKEYKCKVSNKALPAPIEKTISKAKGQPREPQVYTLPPSRDELTKNQVSLTCLVKGFYPSDIAVEWESNGQPENNYKTTPPVLDSDGSFFLYSKLTVDKSRWQQGNVFSCSVMHEALHNHYTQKSLSLSPGK

SEQ ID NO: 23 - protein, 119 aa, artificial sequence
QVQLVQSGAEVKKPGASVKVSCKASGYTFTTHYMYWVRQAPGQGLEWIGGINPSNGATNFNEKFKTKATLTVDKSTSTAYMELSSLRSEDTAVYYCTRVGGLSYTMDYWGQGTLVTVSS

SEQ ID NO: 24 - protein, 449 aa, artificial sequence
QVQLVQSGAEVKKPGASVKVSCKASGYTFTTHYMYWVRQAPGQGLEWMGGINPSNGATNFNEKFKTRVTMTVDKSTSTAYMELSSLRSEDTAVYYCTRVGGLSYTMDYWGQGTLVTVSSASTKGPSVFPLAPSSKSTSGGTAALGCLVKDYFPEPVTVSWNSGALTSGVHTFPAVLQSSGLYSLSSVVTVPSSSLGTQTYICNVNHKPSNTKVDKKVEPKSCDKTHTCPPCPAPELLGGPSVFLFPPKPKDTLMISRTPEVTCVVVDVSHEDPEVKFNWYVDGVEVHNAKTKPREEQYNSTYRVVSVLTVLHQDWLNGKEYKCKVSNKALPAPIEKTISKAKGQPREPQVYTLPPSRDELTKNQVSLTCLVKGFYPSDIAVEWESNGQPENNYKTTPPVLDSDGSFFLYSKLTVDKSRWQQGNVFSCSVMHEALHNHYTQKSLSLSPGK

SEQ ID NO: 25 - protein, 119 aa, artificial sequence
QVQLVQSGAEVKKPGASVKVSCKASGYTFTTHYMYWVRQAPGQGLEWMGGINPSNGATNFNEKFKTRVTMTVDKSTSTAYMELSSLRSEDTAVYYCTRVGGLSYTMDYWGQGTLVTVSS

SEQ ID NO: 26 - protein, 449 aa, artificial sequence
QVQLVQSGAEVKKPGASVKVSCKASGYTFTTHYMYWVRQAPGQGLEWIGGINPSNGATNFNEKFKTRVTLTVDKSISTAYMELSRLRSDDTAVYYCTRVGGLSYTMDYWGQGTLVTVSSASTKGPSVFPLAPSSKSTSGGTAALGCLVKDYFPEPVTVSWNSGALTSGVHTFPAVLQSSGLYSLSSVVTVPSSSLGTQTYICNVNHKPSNTKVDKKVEPKSCDKTHTCPPCPAPELLGGPSVFLFPPKPKDTLMISRTPEVTCVVVDVSHEDPEVKFNWYVDGVEVHNAKTKPREEQYNSTYRVVSVLTVLHQDWLNGKEYKCKVSNKALPAPIEKTISKAKGQPREPQVYTLPPSRDELTKNQVSLTCLVKGFYPSDIAVEWESNGQPENNYKTTPPVLDSDGSFFLYSKLTVDKSRWQQGNVFSCSVMHEALHNHYTQKSLSLSPGK

SEQ ID NO: 27 - protein, 119 aa, artificial sequence
QVQLVQSGAEVKKPGASVKVSCKASGYTFTTHYMYWVRQAPGQGLEWIGGINPSNGATNFNEKFKTRVTLTVDKSISTAYMELSRLRSDDTAVYYCTRVGGLSYTMDYWGQGTLVTVSS

SEQ ID NO: 28 - protein, 449 aa, artificial sequence
QVQLVQSGAEVKKPGASVKVSCKASGYTFTTHYMYWVKQAPGQGLEWIGGINPSNGATNFNEKFKTKATLTVDKSISTAYMELSRLRSDDTAVYYCTRVGGLSYTMDYWGQGTLVTVSSASTKGPSVFPLAPSSKSTSGGTAALGCLVKDYFPEPVTVSWNSGALTSGVHTFPAVLQSSGLYSLSSVVTVPSSSLGTQTYICNVNHKPSNTKVDKKVEPKSCDKTHTCPPCPAPELLGGPSVFLFPPKPKDTLMISRTPEVTCVVVDVSHEDPEVKFNWYVDGVEVHNAKTKPREEQYNSTYRVVSVLTVLHQDWLNGKEYKCKVSNKALPAPIEKTISKAKGQPREPQVYTLPPSRDELTKNQVSLTCLVKGFYPSDIAVEWESNGQPENNYKTTPPVLDSDGSFFLYSKLTVDKSRWQQGNVFSCSVMHEALHNHYTQKSLSLSPGK

SEQ ID NO: 29 - protein, 119 aa, artificial sequence
QVQLVQSGAEVKKPGASVKVSCKASGYTFTTHYMYWVKQAPGQGLEWIGGINPSNGATNFNEKFKTKATLTVDKSISTAYMELSRLRSDDTAVYYCTRVGGLSYTMDYWGQGTLVTVSS

SEQ ID NO: 30 - protein, 232 aa, artificial sequence
EPKSSDKTHTCPPCPAPEAAGGPSVFLFPPKPKDTLMISRTPEVTCVVVAVSHEDPEVKFNWYVDGVEVHNAKTKPREEQYNSTYRVVSVLTVLHQDWLNGKEYKCKVSNKALAAPIEKTISKAKGQPREPQVCTLPPSRDELTKNQVSLSCAVKGFYPSDIAVEWESNGQPENNYKTTPPVLDSDGSFFLVSKLTVDKSRWQQGNVFSCSVMHEALHNHYTQKSLSLSPGK

SEQ ID NO: 31 - protein, 704 aa, artificial sequence
QVQLVQSGAEVKKPGASVKVSCKASGYTFTTHYMYWVRQAPGQGLEWIGGINPSNGATNFNEKFKTKATLTVDKSTSTAYMELSSLRSEDTAVYYCTRVGGLSYTMDYWGQGTLVTVSSASTKGPSVFPLAPSSKSTSGGTAALGCLVKDYFPEPVTVSWNSGALTSGVHTFPAVLQSSGLYSLSSVVTVPSSSLGTQTYICNVNHKPSNTKVDKKVEPKSCEVQLVESGGGLVQPGGSLKLSCAASGFTFSTYAMNWVRQAPGKGLEWVGRIRSKYNNYATYYADSVKDRFTISRDDSKNTLYLQMNSLKTEDTAVYYCTRHGNFGNSYVSWFAYWGQGTTVTVSSGGGGSGGGGSGGGGSQAVVTQEPSLTVSPGGTVTLTCRSSTGAVTTSNYANWVQQKPGQAPRGLIGGTNKRAPGVPARFSGSLLGGKAALTLSGAQPEDEAEYFCALWYSNLWVFGGGTKLTVLGEPKSSDKTHTCPPCPAPEAAGGPSVFLFPPKPKDTLMISRTPEVTCVVVAVSHEDPEVKFNWYVDGVEVHNAKTKPREEQYNSTYRVVSVLTVLHQDWLNGKEYKCKVSNKALAAPIEKTISKAKGQPREPQVYTLPPCRDELTKNQVSLWCLVKGFYPSDIAVEWESNGQPENNYKTTPPVLDSDGSFFLYSKLTVDKSRWQQGNVFSCSVMHEALHNHYTQKSLSLSPGK

SEQ ID NO: 32 - protein, 449 aa, artificial sequence
QVQLVQSGAEVKKPGASVKVSCKASGYTFTTHYMYWVRQAPGQGLEWIGGINPSSGATNFNEKFKTKATLTVDKSTSTAYMELSSLRSEDTAVYYCTRVGGLSYTMDYWGQGTLVTVSSASTKGPSVFPLAPSSKSTSGGTAALGCLVKDYFPEPVTVSWNSGALTSGVHTFPAVLQSSGLYSLSSVVTVPSSSLGTQTYICNVNHKPSNTKVDKKVEPKSCDKTHTCPPCPAPEAAGGPSVFLFPPKPKDTLMISRTPEVTCVVVAVSHEDPEVKFNWYVDGVEVHNAKTKPREEQYNSTYRVVSVLTVLHQDWLNGKEYKCKVSNKALAAPIEKTISKAKGQPREPQVCTLPPSRDELTKNQVSLSCAVKGFYPSDIAVEWESNGQPENNYKTTPPVLDSDGSFFLVSKLTVDKSRWQQGNVFSCSVMHEALHNHYTQKSLSLSPGK

SEQ ID NO: 33 - protein, 449 aa, artificial sequence
QVQLVQSGAEVKKPGASVKVSCKASGYTFTTHYMYWVRQAPGQGLEWIGGINPSNGATNFNEKFKTKATLTVDKSTSTAYMELSSLRSEDTAVYYCTRVGGLSYTMDYWGQGTLVTVSSASTKGPSVFPLAPSSKSTSGGTAALGCLVKDYFPEPVTVSWNSGALTSGVHTFPAVLQSSGLYSLSSVVTVPSSSLGTQTYICNVNHKPSNTKVDKKVEPKSCDKTHTCPPCPAPEAAGGPSVFLFPPKPKDTLMISRTPEVTCVVVAVSHEDPEVKFNWYVDGVEVHNAKTKPREEQYNSTYRVVSVLTVLHQDWLNGKEYKCKVSNKALAAPIEKTISKAKGQPREPQVCTLPPSRDELTKNQVSLSCAVKGFYPSDIAVEWESNGQPENNYKTTPPVLDSDGSFFLVSKLTVDKSRWQQGNVFSCSVMHEALHNHYTQKSLSLSPGK

SEQ ID NO: 34 - protein, 704 aa, artificial sequence
QVQLVQSGAEVKKPGASVKVSCKASGYTFTTHYMYWVRQAPGQGLEWIGGINPSSGATNFNEKFKTKATLTVDKSTSTAYMELSSLRSEDTAVYYCTRVGGLSYTMDYWGQGTLVTVSSASTKGPSVFPLAPSSKSTSGGTAALGCLVKDYFPEPVTVSWNSGALTSGVHTFPAVLQSSGLYSLSSVVTVPSSSLGTQTYICNVNHKPSNTKVDKKVEPKSCEVQLVESGGGLVQPGGSLKLSCAASGFTFSTYAMNWVRQAPGKGLEWVGRIRSKYNNYATYYADSVKDRFTISRDDSKNTLYLQMNSLKTEDTAVYYCTRHGNFGNSYVSWFAYWGQGTTVTVSSGGGGSGGGGSGGGGSQAVVTQEPSLTVSPGGTVTLTCRSSTGAVTTSNYANWVQQKPGQAPRGLIGGTNKRAPGVPARFSGSLLGGKAALTLSGAQPEDEAEYFCALWYSNLWVFGGGTKLTVLGEPKSSDKTHTCPPCPAPEAAGGPSVFLFPPKPKDTLMISRTPEVTCVVVAVSHEDPEVKFNWYVDGVEVHNAKTKPREEQYNSTYRVVSVLTVLHQDWLNGKEYKCKVSNKALAAPIEKTISKAKGQPREPQVYTLPPCRDELTKNQVSLWCLVKGFYPSDIAVEWESNGQPENNYKTTPPVLDSDGSFFLYSKLTVDKSRWQQGNVFSCSVMHEALHNHYTQKSLSLSPGK

SEQ ID NO: 35 - protein, 706 aa, artificial sequence
QVQLVQSGAEVKKPGASVKVSCKASGYTFTTHYMYWVRQAPGQGLEWIGGINPSNEATNFNEKFKTKATLTVDKSTSTAYMELSSLRSEDTAVYYCTRVGGLSYTMDYWGQGTLVTVSSASTKGPSVFPLAPSSKSTSGGTAALGCLVKDYFPEPVTVSWNSGALTSGVHTFPAVLQSSGLYSLSSVVTVPSSSLGTQTYICNVNHKPSNTKVDKKVEPKSCEVQLVESGGGLVQPGGSLKLSCAASGFTFSTYAMNWVRQAPGKGLEWVGRIRSKYNNYATYYADSVKDRFTISRDDSKNTLYLQMNSLKTEDTAVYYCTRHGNFGNSYVSWFAYWGQGTTVTVSSGGGGSGGGGSGGGGSQAVVTQEPSLTVSPGGTVTLTCRSSTGAVTTSNYANWVQQKPGQAPRGLIGGTNKRAPGVPARFSGSLLGGKAALTLSGAQPEDEAEYFCALWYSNLWVFGGGTKLTVLGEPKSSDKTHTCPPCPAPEAAGGPSVFLFPPKPKDTLMISRTPEVTCVVVAVSHEDPEVKFNWYVDGVEVHNAKTKPREEQYNSTYRVVSVLTVLHQDWLNGKEYKCKVSNKALAAPIEKTISKAKGQPREPQVYTLPPCRDELTKNQVSLWCLVKGFYPSDIAVEWESNGQPENNYKTTPPVLDSDGSFFLYSKLTVDKSRWQQGNVFSCSVMHEALHNHYTQKSLSLSPGKGE

SEQ ID NO: 36 - protein, 449 aa, artificial sequence
QVQLVQSGAEVKKPGASVKVSCKASGYTFTTHYMYWVRQAPGQGLEWIGGINPSNEATNFNEKFKTKATLTVDKSTSTAYMELSSLRSEDTAVYYCTRVGGLSYTMDYWGQGTLVTVSSASTKGPSVFPLAPSSKSTSGGTAALGCLVKDYFPEPVTVSWNSGALTSGVHTFPAVLQSSGLYSLSSVVTVPSSSLGTQTYICNVNHKPSNTKVDKKVEPKSCDKTHTCPPCPAPEAAGGPSVFLFPPKPKDTLMISRTPEVTCVVVAVSHEDPEVKFNWYVDGVEVHNAKTKPREEQYNSTYRVVSVLTVLHQDWLNGKEYKCKVSNKALAAPIEKTISKAKGQPREPQVCTLPPSRDELTKNQVSLSCAVKGFYPSDIAVEWESNGQPENNYKTTPPVLDSDGSFFLVSKLTVDKSRWQQGNVFSCSVMHEALHNHYTQKSLSLSPGK

SEQ ID NO: 37 - protein, 482 aa, artificial sequence
EVQLVESGGGLVQPGGSLKLSCAASGFTFSTYAMNWVRQAPGKGLEWVGRIRSKYNNYATYYADSVKDRFTISRDDSKNTLYLQMNSLKTEDTAVYYCTRHGNFGNSYVSWFAYWGQGTTVTVSSGGGGSGGGGSGGGGSQAVVTQEPSLTVSPGGTVTLTCRSSTGAVTTSNYANWVQQKPGQAPRGLIGGTNKRAPGVPARFSGSLLGGKAALTLSGAQPEDEAEYFCALWYSNLWVFGGGTKLTVLGEPKSSDKTHTCPPCPAPEAAGGPSVFLFPPKPKDTLMISRTPEVTCVVVAVSHEDPEVKFNWYVDGVEVHNAKTKPREEQYNSTYRVVSVLTVLHQDWLNGKEYKCKVSNKALAAPIEKTISKAKGQPREPQVYTLPPCRDELTKNQVSLWCLVKGFYPSDIAVEWESNGQPENNYKTTPPVLDSDGSFFLYSKLTVDKSRWQQGNVFSCSVMHEALHNHYTQKSLSLSPGK

SEQ ID NO: 38 - protein, 119 aa, artificial sequence
QVQLVQSGAEVKKPGASVKVSCKASGYTFTTHYMYWVRQAPGQGLEWIGGINPSSGATNFNEKFKTKATLTVDKSTSTAYMELSSLRSEDTAVYYCTRVGGLSYTMDYWGQGTLVTVSS

SEQ ID NO: 39 - protein, 17 aa, artificial sequence
GINPSSGATNFNEKFKT

SEQ ID NO: 40 - protein, 121 aa, artificial sequence
QVQLVQSGAEVKKPGASVKVSCKASGYTFTTHYMYWVRQAPGQGLEWIGGINPSNEATNFNEKFKTKATLTVDKSTSTAYMELSSLRSEDTAVYYCTRVGGLSYTMDYWGQGTLVTVSSGE

SEQ ID NO: 41 - protein, 17 aa, artificial sequence
GINPSNEATNFNEKFKT

SEQ ID NO: 42 - protein, 227 aa, artificial sequence
DKTHTCPPCPAPEAAGGPSVFLFPPKPKDTLMISRTPEVTCVVVAVSHEDPEVKFNWYVDGVEVHNAKTKPREEQYNSTYRVVSVLTVLHQDWLNGKEYKCKVSNKALAAPIEKTISKAKGQPREPQVCTLPPSRDELTKNQVSLSCAVKGFYPSDIAVEWESNGQPENNYKTTPPVLDSDGSFFLVSKLTVDKSRWQQGNVFSCSVMHEALHNHYTQKSLSLSPGK

SEQ ID NO: 43 - protein, 232 aa, artificial sequence
EPKSSDKTHTCPPCPAPEAAGGPSVFLFPPKPKDTLMISRTPEVTCVVVAVSHEDPEVKFNWYVDGVEVHNAKTKPREEQYNSTYRVVSVLTVLHQDWLNGKEYKCKVSNKALAAPIEKTISKAKGQPREPQVYTLPPCRDELTKNQVSLWCLVKGFYPSDIAVEWESNGQPENNYKTTPPVLDSDGSFFLYSKLTVDKSRWQQGNVFSCSVMHEALHNHYTQKSLSLSPGK

SEQ ID NO: 44 - protein, 103 aa, artificial sequence
ASTKGPSVFPLAPSSKSTSGGTAALGCLVKDYFPEPVTVSWNSGALTSGVHTFPAVLQSSGLYSLSSVVTVPSSSLGTQTYICNVNHKPSNTKVDKKVEPKSC

SEQ ID NO: 45 - protein, 330 aa, artificial sequence
ASTKGPSVFPLAPSSKSTSGGTAALGCLVKDYFPEPVTVSWNSGALTSGVHTFPAVLQSSGLYSLSSVVTVPSSSLGTQTYICNVNHKPSNTKVDKKVEPKSCDKTHTCPPCPAPEAAGGPSVFLFPPKPKDTLMISRTPEVTCVVVAVSHEDPEVKFNWYVDGVEVHNAKTKPREEQYNSTYRVVSVLTVLHQDWLNGKEYKCKVSNKALAAPIEKTISKAKGQPREPQVYTLPPSRDELTKNQVSLTCLVKGFYPSDIAVEWESNGQPENNYKTTPPVLDSDGSFFLYSKLTVDKSRWQQGNVFSCSVMHEALHNHYTQKSLSLSPGK

SEQ ID NO: 46 - protein, 227 aa, artificial sequence
DKTHTCPPCPAPEAAGGPSVFLFPPKPKDTLMISRTPEVTCVVVAVSHEDPEVKFNWYVDGVEVHNAKTKPREEQYNSTYRVVSVLTVLHQDWLNGKEYKCKVSNKALAAPIEKTISKAKGQPREPQVYTLPPSRDELTKNQVSLTCLVKGFYPSDIAVEWESNGQPENNYKTTPPVLDSDGSFFLYSKLTVDKSRWQQGNVFSCSVMHEALHNHYTQKSLSLSPGK

SEQ ID NO: 47 - protein, 105 aa, artificial sequence
GQPKAAPSVTLFPPSSEELQANKATLVCLISDFYPGAVTVAWKADSSPVKAGVETTTPSKQSNNKYAASSYLSLTPEQWKSHRSYSCQVTHEGSTVEKTVAPTEC

SEQ ID NO: 48 - protein, 330 aa, artificial sequence [sequence omitted]

SEQ ID NO: 49 - protein, 227 aa, artificial sequence
DKTHTCPPCPAPELLGGPSVFLFPPKPKDTLMISRTPEVTCVVVDVSHEDPEVKFNWYVDGVEVHNAKTKPREEQYNSTYRVVSVLTVLHQDWLNGKEYKCKVSNKALPAPIEKTISKAKGQPREPQVYTLPPSRDELTKNQVSLTCLVKGFYPSDIAVEWESNGQPENNYKTTPPVLDSDGSFFLYSKLTVDKSRWQQGNVFSCSVMHEALHNHYTQKSLSLSPGK

SEQ ID NO: 50 - protein, 107 aa, artificial sequence [sequence omitted]

SEQ ID NO: 51 - protein, 455 aa, artificial sequence
EVQLLESGGGLVQPGGSLRLSCAASGFTFSTYAMNWVRQAPGKGLEWVSRIRSKYNNYATYYADSVKGRFTISRDDSKNTLYLQMNSLRAEDTAVYYCVRHGNFGNSYVSWFAYWGQGTLVTVSSASTKGPSVFPLAPSSKSTSGGTAALGCLVKDYFPEPVTVSWNSGALTSGVHTFPAVLQSSGLYSLSSVVTVPSSSLGTQTYICNVNHKPSNTKVDKKVEPKSCDKTHTCPPCPAPEAAGGPSVFLFPPKPKDTLMISRTPEVTCVVVAVSHEDPEVKFNWYVDGVEVHNAKTKPREEQYNSTYRVVSVLTVLHQDWLNGKEYKCKVSNKALAAPIEKTISKAKGQPREPQVYTLPPSRDELTKNQVSLTCLVKGFYPSDIAVEWESNGQPENNYKTTPPVLDSDGSFFLYSKLTVDKSRWQQGNVFSCSVMHEALHNHYTQKSLSLSPGK

SEQ ID NO: 52 - protein, 214 aa, artificial sequence
QAVVTQEPSLTVSPGGTVTLTCGSSTGAVTTSNYANWVQEKPGQAFRGLIGGTNKRAPGTPARFSGSLLGGKAALTLSGAQPEDEAEYYCALWYSNLWVFGGGTKLTVLGQPKAAPSVTLFPPSSEELQANKATLVCLISDFYPGAVTVAWKADSSPVKAGVETTTPSKQSNNKYAASSYLSLTPEQWKSHRSYSCQVTHEGSTVEKTVAPTEC

SEQ ID NO: 53 - protein, 452 aa, artificial sequence
EVQLVESGGGLVQPGGSLRLSCAASGFTFNTYAMNWVRQAPGKGLEWVARIRSKYNNYATYYAASVKGRFTISRDDSKNSLYLQMNSLKTEDTAVYYCARHGNFGNSYVSWFAYWGQGTLVTVSSASTKGPSVFPLAPCSRSTSESTAALGCLVKDYFPEPVTVSWNSGALTSGVHTFPAVLQSSGLYSLSSVVTVPSSSLGTKTYTCNVDHKPSNTKVDKRVESKYGPPCPPCPAPEAAGGPSVFLFPPKPKDTLMISRTPEVTCVVVDVSQEDPEVQFNWYVDGVEVHNAKTKPREEQFNSTYRVVSVLTVLHQDWLNGKEYKCKVSNKGLPSSIEKTISKAKGQPREPQVYTLPPSQEEMTKNQVSLTCLVKGFYPSDIAVEWESNGQPENNYKTTPPVLDSDGSFLLYSKLTVDKSRWQEGNVFSCSVMHEALHNHYTQKSLSLSLGK

SEQ ID NO: 54 - protein, 214 aa, artificial sequence
QTVVTQEPSLTVSPGGTVTLTCRSSTGAVTTSNYANWVQQKPGQAPRGLIGGTNKRAPGTPARFSGSLLGGKAALTLSGVQPEDEAEYYCALWYSNLWVFGGGTKLTVLGQPKAAPSVTLFPPSSEELQANKATLVCLISDFYPGAVTVAWKADSSPVKAGVETTTPSKQSNNKYAASSYLSLTPEQWKSHRSYSCQVTHEGSTVEKTVAPTEC

SEQ ID NO: 55 - protein, 445 aa, artificial sequence
QVQLVQSGAEVKKPGASVKVSCKASGYSFTGYTMNWVRQAPGQGLEWMGLINPYNSDTNYAQKLQGRVTMTTDTSTSTAYMELRSLRSDDTAVYYCARVALRVALDYWGQGTLVTVSSASTKGPSVFPLAPCSRSTSESTAALGCLVKDYFPEPVTVSWNSGALTSGVHTFPAVLQSSGLYSLSSVVTVPSSSLGTKTYTCNVDHKPSNTKVDKRVESKYGPPCPPCPAPEAAGGPSVFLFPPKPKDTLMISRTPEVTCVVVDVSQEDPEVQFNWYVDGVEVHNAKTKPREEQFNSTYRVVSVLTVLHQDWLNGKEYKCKVSNKGLPSSIEKTISKAKGQPREPQVYTLPPSQEEMTKNQVSLTCLVKGFYPSDIAVEWESNGQPENNYKTTPPVLDSDGSFFLYSRLTVDKSRWQEGNVFSCSVMHEALHNHYTQKSLSLSLGK

SEQ ID NO: 56 - protein, 214 aa, artificial sequence
DIQMTQSPSSLSASVGDRVTITCKASQNVATHVGWYQQKPGKAPKRLIYSASYRYSGVPSRFSGSGSGTEFTLTISNLQPEDFATYYCQQYNRYPYTFGQGTKLEIKRTVAAPSVFIFPPSDEQLKSGTASVVCLLNNFYPREAKVQWKVDNALQSGNSQESVTEQDSKDSTYSLSSTLTLSKADYEKHKVYACEVTHQGLSSPVTKSFNRGEC

SEQ ID NO: 57 - protein, 345 aa, artificial sequence
MYKDCIESTGDYFLLCDAEGPWGIILESLAILGIVVTILLLLAFLFLMRKIQDCSQWNVLPTQLLFLLSVLGLFGLAFAFIIELNQQTAPVRYFLFGVLFALCFSCLLAHASNLVKLVRGCVSFSWTTILCIAIGCSLLQIIIATEYVTLIMTRGMMFVNMTPCQLNVDFVVLLVYVLFLMALTFFVSKATFCGPCENWKQHGRLIFITVLFSIIIWVVWISMLLRGNPQFQRQPQWDDPVVCIALVTNAWVFLLLYIVPELCILYRSCRQECPLQGNACPVTAYQHSFQVENQELSRARDSDGAEEDVALTSYGTPIQPQTVDPTQECFIPQAKLSPQQDAGGV

SEQ ID NO: 58 - protein, 344 aa, artificial sequence
MYKDCIESTGDYFLPCDSEGPWGIILESLAILGIVVTILLLLAFLFLMRKIQDCSQWNVLPTQLLFLLSVLGLFGLAFAFIIQLNQQTAPVRYFLFGVLFALCFSCLLAHASNLVKLVRGRVSFSWTTILCIAIGCSLLQVIIAIEYVTLIMTRGMMFVHMTPYQLNVDFVVLLVYVLFLMALTFFVSKATFCGPCENWKQHGRLIFITVLFSIIIWVVWISMLLRGNPQFQRQPQWDDPVVCIALVTNAWVFLLLYIVPELCILYRSCRQECPSQGHACPVTAYQRSFQVENQELSRARDSDGAEEDVALTSFGTPIQPQTVDPTQECFIPRAKLSPQQDAGV

SEQ ID NO: 59 - protein, 232 aa, artificial sequence
EPKSCDKTHTCPPCPAPEAAGGPSVFLFPPKPKDTLMISRTPEVTCVVVAVSHEDPEVKFNWYVDGVEVHNAKTKPREEQYNSTYRVVSVLTVLHQDWLNGKEYKCKVSNKALAAPIEKTISKAKGQPREPQVCTLPPSRDELTKNQVSLSCAVKGFYPSDIAVEWESNGQPENNYKTTPPVLDSDGSFFLVSKLTVDKSRWQQGNVFSCSVMHEALHNHYTQKSLSLSPGK

SEQ ID NO: 60 - protein, 449 aa, artificial sequence
QVQLQQPGAELVKPGASVKLSCKASGYTFTTHYMYWVKQRPGQGLEWIGGINPSNGATNFNEKFKTKATLTVDKSSSTAYMQLSSLTSEDSAVYYCTRVGGLSYTMDYWGQGTSVTVSSASTKGPSVFPLAPSSKSTSGGTAALGCLVKDYFPEPVTVSWNSGALTSGVHTFPAVLQSSGLYSLSSVVTVPSSSLGTQTYICNVNHKPSNTKVDKKVEPKSCDKTHTCPPCPAPELLGGPSVFLFPPKPKDTLMISRTPEVTCVVVDVSHEDPEVKFNWYVDGVEVHNAKTKPREEQYNSTYRVVSVLTVLHQDWLNGKEYKCKVSNKALPAPIEKTISKAKGQPREPQVYTLPPSRDELTKNQVSLTCLVKGFYPSDIAVEWESNGQPENNYKTTPPVLDSDGSFFLYSKLTVDKSRWQQGNVFSCSVMHEALHNHYTQKSLSLSPGK

SEQ ID NO: 61 - protein, 220 aa, artificial sequence
DIVMSQSPSSLAVSVGEKVSMSCKSSQSLLYSSNQKNYLAWYQQKPGQSPKLLIYWASTRESGVPDRFTGSGYGTDFTLTISSMKAEDLAVYYCQQYYSYPRTFGGGTKLDIKRTVAAPSVFIFPPSDEQLKSGTASVVCLLNNFYPREAKVQWKVDNALQSGNSQESVTEQDSKDSTYSLSSTLTLSKADYEKHKVYACEVTHQGLSSPVTKSFNRGEC

SEQ ID NO: 62 - protein, 119 aa, artificial sequence
QVQLQQPGAELVKPGASVKLSCKASGYTFTTHYMYWVKQRPGQGLEWIGGINPSNGATNFNEKFKTKATLTVDKSSSTAYMQLSSLTSEDSAVYYCTRVGGLSYTMDYWGQGTSVTVSS

SEQ ID NO: 63 - protein, 113 aa, artificial sequence
DIVMSQSPSSLAVSVGEKVSMSCKSSQSLLYSSNQKNYLAWYQQKPGQSPKLLIYWASTRESGVPDRFTGSGYGTDFTLTISSMKAEDLAVYYCQQYYSYPRTFGGGTKLDIK

SEQ ID NO: 64 - protein, 5 aa, artificial sequence
THYMY

SEQ ID NO: 65 - protein, 17 aa, artificial sequence
GINPSNGATNFNEKFKT

SEQ ID NO: 66 - protein, 10 aa, artificial sequence
VGGLSYTMDY

SEQ ID NO: 67 - protein, 17 aa, artificial sequence
KSSQSLLYSSNQKNYLA

SEQ ID NO: 68 - protein, 7 aa, artificial sequence
WASTRES

SEQ ID NO: 69 - protein, 9 aa, artificial sequence
QQYYSYPRT

SEQ ID NO: 70 - protein, 446 aa, artificial sequence
DVQLVESGGGLVQPRGSRKLSCAASGFTFSSFGMHWVRQAPEKGLEWVAYISSDSNTIYYADTVQGRFTISRDNPKNTLFLQMTRLRSEDTAMYYCARNPWYFDVWGAGTTVTVSSASTKGPSVFPLAPSSKSTSGGTAALGCLVKDYFPEPVTVSWNSGALTSGVHTFPAVLQSSGLYSLSSVVTVPSSSLGTQTYICNVNHKPSNTKVDKKVEPKSCDKTHTCPPCPAPELLGGPSVFLFPPKPKDTLMISRTPEVTCVVVDVSHEDPEVKFNWYVDGVEVHNAKTKPREEQYNSTYRVVSVLTVLHQDWLNGKEYKCKVSNKALPAPIEKTISKAKGQPREPQVYTLPPSRDELTKNQVSLTCLVKGFYPSDIAVEWESNGQPENNYKTTPPVLDSDGSFFLYSKLTVDKSRWQQGNVFSCSVMHEALHNHYTQKSLSLSPGK

SEQ ID NO: 71 - protein, 219 aa, artificial sequence
DVLMTQTPLSLPVSLGDQVSISCRSSQSIVHSNGNTYLEWFLQKPGQSPKLLIYKVSNRFSGVPDRFSGSGSGTDFTLKISRVEAEDLGIYYCFQGSHIPPTFGGGTKLEIKRTVAAPSVFIFPPSDEQLKSGTASVVCLLNNFYPREAKVQWKVDNALQSGNSQESVTEQDSKDSTYSLSSTLTLSKADYEKHKVYACEVTHQGLSSPVTKSFNRGEC

SEQ ID NO: 72 - protein, 116 aa, artificial sequence
DVQLVESGGGLVQPRGSRKLSCAASGFTFSSFGMHWVRQAPEKGLEWVAYISSDSNTIYYADTVQGRFTISRDNPKNTLFLQMTRLRSEDTAMYYCARNPWYFDVWGAGTTVTVSS

SEQ ID NO: 73 - protein, 112 aa, artificial sequence
DVLMTQTPLSLPVSLGDQVSISCRSSQSIVHSNGNTYLEWFLQKPGQSPKLLIYKVSNRFSGVPDRFSGSGSGTDFTLKISRVEAEDLGIYYCFQGSHIPPTFGGGTKLEIK

SEQ ID NO: 74 - protein, 5 aa, artificial sequence
SFGMH

SEQ ID NO: 75 - protein, 17 aa, artificial sequence
YISSDSNTIYYADTVQG

SEQ ID NO: 76 - protein, 7 aa, artificial sequence
NPWYFDV

SEQ ID NO: 77 - protein, 16 aa, artificial sequence
RSSQSIVHSNGNTYLE

SEQ ID NO: 78 - protein, 7 aa, artificial sequence
KVSNRFS

SEQ ID NO: 79 - protein, 9 aa, artificial sequence
FQGSHIPPT

SEQ ID NO: 80 - protein, 446 aa, artificial sequence
QVQLQQPGAELVKPGSSVKLSCKASGYTFTTYWMEWVKQRPGQGLEWIGEINPNNGRSNYNEKFQTKATLTVDKSSSTAYMQFSSLTSEDSAVYYCARERAGLTYWGQGTLVIVSAASTKGPSVFPLAPSSKSTSGGTAALGCLVKDYFPEPVTVSWNSGALTSGVHTFPAVLQSSGLYSLSSVVTVPSSSLGTQTYICNVNHKPSNTKVDKKVEPKSCDKTHTCPPCPAPELLGGPSVFLFPPKPKDTLMISRTPEVTCVVVDVSHEDPEVKFNWYVDGVEVHNAKTKPREEQYNSTYRVVSVLTVLHQDWLNGKEYKCKVSNKALPAPIEKTISKAKGQPREPQVYTLPPSRDELTKNQVSLTCLVKGFYPSDIAVEWESNGQPENNYKTTPPVLDSDGSFFLYSKLTVDKSRWQQGNVFSCSVMHEALHNHYTQKSLSLSPGK

SEQ ID NO: 81 - protein, 219 aa, artificial sequence
DVVMTQTPLSLPVSLGDQASISCRSSQSLVHSNGNTYLHWYLQKPGQSPKLLIYKVSNRFSGVPDRFGGSGSGTDFTLKISRVEAEDLGVYFCSQSTHFPYTFGGGTKLEIKRTVAAPSVFIFPPSDEQLKSGTASVVCLLNNFYPREAKVQWKVDNALQSGNSQESVTEQDSKDSTYSLSSTLTLSKADYEKHKVYACEVTHQGLSSPVTKSFNRGEC

SEQ ID NO: 82 - protein, 116 aa, artificial sequence
QVQLQQPGAELVKPGSSVKLSCKASGYTFTTYWMEWVKQRPGQGLEWIGEINPNNGRSNYNEKFQTKATLTVDKSSSTAYMQFSSLTSEDSAVYYCARERAGLTYWGQGTLVIVSA

SEQ ID NO: 83 - protein, 112 aa, artificial sequence
DVVMTQTPLSLPVSLGDQASISCRSSQSLVHSNGNTYLHWYLQKPGQSPKLLIYKVSNRFSGVPDRFGGSGSGTDFTLKISRVEAEDLGVYFCSQSTHFPYTFGGGTKLEIK

SEQ ID NO: 84 - protein, 5 aa, artificial sequence
TYWME

SEQ ID NO: 85 - protein, 17 aa, artificial sequence
EINPNNGRSNYNEKFQT

SEQ ID NO: 86 - protein, 7 aa, artificial sequence
ERAGLTY

SEQ ID NO: 87 - protein, 16 aa, artificial sequence
RSSQSLVHSNGNTYLH

SEQ ID NO: 88 - protein, 9 aa, artificial sequence
SQSTHFPYT

SEQ ID NO: 89 - protein, 227 aa, artificial sequence
DKTHTCPPCPAPEAAGGPSVFLFPPKPKDTLMISRTPEVTCVVVAVSHEDPEVKFNWYVDGVEVHNAKTKPREEQYNSTYRVVSVLTVLHQDWLNGKEYKCKVSNKALAAPIEKTISKAKGQPREPQVYTLPPCRDELTKNQVSLWCLVKGFYPSDIAVEWESNGQPENNYKTTPPVLDSDGSFFLYSKLTVDKSRWQQGNVFSCSVMHEALHNHYTQKSLSLSPGK

SEQ ID NO: 90 - protein, 125 aa, artificial sequence
EVQLVESGGGLVQPKGSLKLSCAASGFTFNTYAMNWVRQAPGKGLEWVARIRSKYNNYATYYADSVKDRFTISRDDSQSILYLQMNNLKTEDTAMYYCVRHGNFGNSYVSWFAYWGQGTLVTVSS

SEQ ID NO: 91 - protein, 109 aa, artificial sequence
QAVVTQESALTTSPGETVTLTCRSSTGAVTTSNYANWVQEKPDHLFTGLIGGTNKRAPGVPARFSGSLIGDKAALTITGAQTEDEAIYFCALWYSNLWVFGGGTKLTVL

SEQ ID NO: 92 - protein, 120 aa, artificial sequence
EVQLQQSGPELVKPGASVKISCKASGYTFTDYNIHWVKQSHGKILEWIGYIYPYNGVSDYNQNFKSKATLIVDNSSNTAYMELRSLTSEDSAVYYCARWDFGSGYYFDYWGQGTTLTVSS

SEQ ID NO: 93 - protein, 5 aa, artificial sequence
DYNIH

SEQ ID NO: 94 - protein, 17 aa, artificial sequence
YIYPYNGVSDYNQNFKS

SEQ ID NO: 95 - protein, 11 aa, artificial sequence
WDFGSGYYFDY

SEQ ID NO: 96 - protein, 106 aa, artificial sequence
QIVLSQSPAILFASPGETVTMTCRASSSVIYMCWNQQKPGSSPKPWIYGTSTLASGVPTRFSGSGSGTSYSLTISRVEAEDAATYYCQQWSSNPFTFGSGTKLEIK

SEQ ID NO: 97 - protein, 10 aa, artificial sequence
RASSSVIYMC

SEQ ID NO: 98 - protein, 7 aa, artificial sequence
GTSTLAS

SEQ ID NO: 99 - protein, 9 aa, artificial sequence
QQWSSNPFT

SEQ ID NO: 100 - protein, 105 aa, artificial sequence
QIVLSQSPAILFASPGETVTMTCRASSSVIYMAWNQQKPGSSPKPWIYGTSTLASGVPTRFSGSGSGTSYSLTISRVEAEDAATYYCQQWSSNPFTFGSGTKLEI

SEQ ID NO: 101 - protein, 10 aa, artificial sequence
RASSSVIYMA

SEQ ID NO: 102 - protein, 106 aa, artificial sequence
QIVLSQSPAILFASPGETVTMTCRASSSVIYMSWNQQKPGSSPKPWIYGTSTLASGVPTRFSGSGSGTSYSLTISRVEAEDAATYYCQQWSSNPFTFGSGTKLEIK

SEQ ID NO: 103 - protein, 10 aa, artificial sequence
RASSSVIYMS

SEQ ID NO: 104 - protein, 455 aa, artificial sequence
EVQLVESGGGLVQPKGSLKLSCAASGFTFNTYAMNWVRQAPGKGLEWVARIRSKYNNYATYYADSVKDRFTISRDDSQSILYLQMNNLKTEDTAMYYCVRHGNFGNSYVSWFAYWGQGTLVTVSSASTKGPSVFPLAPSSKSTSGGTAALGCLVKDYFPEPVTVSWNSGALTSGVHTFPAVLQSSGLYSLSSVVTVPSSSLGTQTYICNVNHKPSNTKVDKKVEPKSCDKTHTCPPCPAPEAAGGPSVFLFPPKPKDTLMISRTPEVTCVVVAVSHEDPEVKFNWYVDGVEVHNAKTKPREEQYNSTYRVVSVLTVLHQDWLNGKEYKCKVSNKALAAPIEKTISKAKGQPREPQVYTLPPSRDELTKNQVSLTCLVKGFYPSDIAVEWESNGQPENNYKTTPPVLDSDGSFFLYSKLTVDKSRWQQGNVFSCSVMHEALHNHYTQKSLSLSPGK

SEQ ID NO: 105 - protein, 214 aa, artificial sequence
QAVVTQESALTTSPGETVTLTCRSSTGAVTTSNYANWVQEKPDHLFTGLIGGTNKRAPGVPARFSGSLIGDKAALTITGAQTEDEAIYFCALWYSNLWVFGGGTKLTVLGQPKAAPSVTLFPPSSEELQANKATLVCLISDFYPGAVTVAWKADSSPVKAGVETTTPSKQSNNKYAASSYLSLTPEQWKSHRSYSCQVTHEGSTVEKTVAPTEC

SEQ ID NO: 106 - protein, 450 aa, artificial sequence
EVQLQQSGPELVKPGASVKISCKASGYTFTDYNIHWVKQSHGKILEWIGYIYPYNGVSDYNQNFKSKATLIVDNSSNTAYMELRSLTSEDSAVYYCARWDFGSGYYFDYWGQGTTLTVSSASTKGPSVFPLAPSSKSTSGGTAALGCLVKDYFPEPVTVSWNSGALTSGVHTFPAVLQSSGLYSLSSVVTVPSSSLGTQTYICNVNHKPSNTKVDKKVEPKSCDKTHTCPPCPAPEAAGGPSVFLFPPKPKDTLMISRTPEVTCVVVAVSHEDPEVKFNWYVDGVEVHNAKTKPREEQYNSTYRVVSVLTVLHQDWLNGKEYKCKVSNKALAAPIEKTISKAKGQPREPQVYTLPPSRDELTKNQVSLTCLVKGFYPSDIAVEWESNGQPENNYKTTPPVLDSDGSFFLYSKLTVDKSRWQQGNVFSCSVMHEALHNHYTQKSLSLSPGK

SEQ ID NO: 107 - protein, 213 aa, artificial sequence
QIVLSQSPAILFASPGETVTMTCRASSSVIYMCWNQQKPGSSPKPWIYGTSTLASGVPTRFSGSGSGTSYSLTISRVEAEDAATYYCQQWSSNPFTFGSGTKLEIKRTVAAPSVFIFPPSDEQLKSGTASVVCLLNNFYPREAKVQWKVDNALQSGNSQESVTEQDSKDSTYSLSSTLTLSKADYEKHKVYACEVTHQGLSSPVTKSFNRGEC

SEQ ID NO: 108 - protein, 213 aa, artificial sequence
QIVLSQSPAILFASPGETVTMTCRASSSVIYMAWNQQKPGSSPKPWIYGTSTLASGVPTRFSGSGSGTSYSLTISRVEAEDAATYYCQQWSSNPFTFGSGTKLEIKRTVAAPSVFIFPPSDEQLKSGTASVVCLLNNFYPREAKVQWKVDNALQSGNSQESVTEQDSKDSTYSLSSTLTLSKADYEKHKVYACEVTHQGLSSPVTKSFNRGEC

SEQ ID NO: 109 - protein, 213 aa, artificial sequence
QIVLSQSPAILFASPGETVTMTCRASSSVIYMSWNQQKPGSSPKPWIYGTSTLASGVPTRFSGSGSGTSYSLTISRVEAEDAATYYCQQWSSNPFTFGSGTKLEIKRTVAAPSVFIFPPSDEQLKSGTASVVCLLNNFYPREAKVQWKVDNALQSGNSQESVTEQDSKDSTYSLSSTLTLSKADYEKHKVYACEVTHQGLSSPVTKSFNRGEC

SEQ ID NO: 110 - protein, 647 aa, artificial sequence
GSRKFNTTERVLQGLLRPLFKNTSVGPLYSGCRLTLLRPEKDGEATGVDAICTHRPDPTGPGLDREQLYLELSQLTHSITELGPYTLDRDSLYVNGFTHRSSVPTTSTGVVSEEPFTLNFTINNLRYMADMGQPGSLKFNITDNVMQHLLSPLFQRSSLGARYTGCRVIALRSVKNGAETRVDLLCTYLQPLSGPGLPIKQVFHELSQQTHGITRLGPYSLDKDSLYLNGYNEPGPDEPPTTPKPATTFLPPLSEATTAMGYHLKTLTLNFTISNLQYSPDMGKGSATFNSTEGVLQHLLRPLFQKSSMGPFYLGCQLISLRPEKDGAATGVDTTCTYHPDPVGPGLDIQQLYWELSQLTHGVTQLGFYVLDRDSLFINGYAPQNLSIRGEYQINFHIVNWNLSNPDPTSSEYITLLRDIQDKVTTLYKGSQLHDTFRFCLVTNLTMDSVLVTVKALFSSNLDPSLVEQVFLDKTLNASFHWLGSTYQLVDIHVTEMESSVYQPTSSSSTQHFYLNFTITNLPYSQDKAQPGTTNYQRNKRNIEDALNQLFRNSSIKSYFSDCQVSTFRSVPNRHHTGVDSLCNFSPLARRVDRVAIYEEFLRMTRNGTQLQNFTLDRSSVLVDGYSPNRNEPLTGNSDLPHHHHHH

SEQ ID NO: 111 - protein, 650 aa, artificial sequence
GSRKFNTTERVLQGLLRPLFKNTSVGPLYSGCRLTLLRPEKDGEATGVDVICTHRPDPTGPGLDREQLYLELSQLTHSITELGPYTLDNDSLFVNGFTHRSSVPTTSTGMVSEEPFTLNFTINNLRYMADMGQPGSLKFNITDNVMQHLLSPLFQRSSVGARYTGCRVIALRSVKNGAKTQVDILCTYLQPLSGPALPIKQVFHELSQQTHGITRLGPYFLDKDSLYLNGYNEPGPDEPPTTPKPATTFLPPLSEATTAMGYHLKTLTLNFTISNLQYSPDMGNGSAAFNSTERVLKHLLRALFQKSSMGPFYLGCQLISLRPEKNGAATGVDTTCTYHTDPVGPGLDIQQLYWELSQLTHGVTQLGFYVLDRDSLFINGYAPQNLSIRGKYQIHFHIVNWNFSNPDPTSSEYIALLRDIQDKVTTLYKGSQLHDTFRYCLVTNLTMDSMLVTVKALFSSDLDPSLVEQVFLDKTLNASSHWLGSTYQLVDIHVTEMEPSVYQPTKPTSSSSTQHFYLNFTITNLPYSQDISQPSTTNYQRNKRNIEDALNQLFRNSSIKSYFSDCQVSTFRSVPNSHHTGVDSLCNFSPLARRVDRVAIYEEFLRMTRNGSQLQNFTLDRSSVLVDGYSPNRNEPLTGNSDLPHHHHHH

SEQ ID NO: 112 - protein, 650 aa, artificial sequence
GSRKFNTTERVLQGLLRPLFKNTSVGPLYSGCRLTLLRPEKDGEATGVDVICTHRPDPTGPGLDREQLYLELSQLTHSITELGPYTLDNDSLFVNGFTHRSSVPTTSTGMVSEEPFTLNFTINNLRYMADMGQPGSLKFNITDNVMQHLLSPLFQRSSVGARYTGCRVIALRSVKNGAKTQVDILCTYLQPLSGPGLPIKQVFHELSQQTHGITRLGPYFLDKDSLYLNGYNEPGPDEPPTTPKPATTFLPPLSEATTAMGYHLKTLTLNFTISNLQYSPDMGNGSAAFNSTERVLKHLLRALFQKSSMGPFYLGCQLISLRPEKNGAATGVDTTCTYHTDPVGPGLDIQQLYWELSQLTHGVTQLGFYVLDRDSLFINGYAPQNLSIRGKYQIHFHIVNWNLGNPDPTSSEYIALLRDIQDKVTTLYKGSRLHDTFCYCLVTNLTMDSMLVTVKALFSSDLDPSLVEQVFLDKTLNASSHWLGSTYQLVDIHVTEMEPSVYQPTKPTSSSSTQHFYLNFTITNLPYSQDISQPSTTNYQRNKRNIEDALNQLFRNSSIKSCFSDCQVSTFRSVPNSHHTGVDSLCNFSPLARRVDRVAIYEEFLRMTRNGSQLQNFTLDRSSVLVDGYSPNRNEPLTGNSDLPHHHHHH

SEQ ID NO: 113 - protein, 120 aa, artificial sequence
QVQLVQSGAEVKKPGASVKVSCKASGYTFTDYNIHWVRQAPGQGLEWMGYIYPYNGVSDYNQNFKSRVTMTTDTSTSTAYMELRSLRSDDTAVYYCARWDFGSGYYFDYWGQGTLVTVSS

SEQ ID NO: 114 - protein, 106 aa, artificial sequence
EIVLTQSPATLSLSPGERATLSCRASSSVIYMSWYQQKPGQAPRLLIYGTSTLASGIPARFSGSGSGTDFTLTISSLEPEDFAVYYCQQWSSNPFTFGQGTKLEIK

SEQ ID NO: 115 - protein, 450 aa, artificial sequence
QVQLVQSGAEVKKPGASVKVSCKASGYTFTDYNIHWVRQAPGQGLEWMGYIYPYNGVSDYNQNFKSRVTMTTDTSTSTAYMELRSLRSDDTAVYYCARWDFGSGYYFDYWGQGTLVTVSSASTKGPSVFPLAPSSKSTSGGTAALGCLVKDYFPEPVTVSWNSGALTSGVHTFPAVLQSSGLYSLSSVVTVPSSSLGTQTYICNVNHKPSNTKVDKKVEPKSCDKTHTCPPCPAPEAAGGPSVFLFPPKPKDTLMISRTPEVTCVVVAVSHEDPEVKFNWYVDGVEVHNAKTKPREEQYNSTYRVVSVLTVLHQDWLNGKEYKCKVSNKALAAPIEKTISKAKGQPREPQVYTLPPSRDELTKNQVSLTCLVKGFYPSDIAVEWESNGQPENNYKTTPPVLDSDGSFFLYSKLTVDKSRWQQGNVFSCSVMHEALHNHYTQKSLSLSPGK

SEQ ID NO: 116 - protein, 213 aa, artificial sequence
EIVLTQSPATLSLSPGERATLSCRASSSVIYMSWYQQKPGQAPRLLIYGTSTLASGIPARFSGSGSGTDFTLTISSLEPEDFAVYYCQQWSSNPFTFGQGTKLEIKRTVAAPSVFIFPPSDEQLKSGTASVVCLLNNFYPREAKVQWKVDNALQSGNSQESVTEQDSKDSTYSLSSTLTLSKADYEKHKVYACEVTHQGLSSPVTKSFNRGEC

SEQ ID NO: 117 - protein, 482 aa, artificial sequence
EVQLVESGGGLVQPGGSLKLSCAASGFTFSTYAMNWVRQAPGKGLEWVGRIRSKYNNYATYYADSVKDRFTISRDDSKNTLYLQMNSLKTEDTAVYYCTRHGNFGNSYVSWFAYWGQGTTVTVSSGGGGSGGGGSGGGGSQAVVTQEPSLTVSPGGTVTLTCRSSTGAVTTSNYANWVQQKPGQAPRGLIGGTNKRAPGVPARFSGSLLGGKAALTLSGAQPEDEAEYFCALWYSNLWVFGGGTKLTVLGEPKSSDKTHTCPPCPAPEAAGGPSVFLFPPKPKDTLMISRTPEVTCVVVAVSHEDPEVKFNWYVDGVEVHNAKTKPREEQYNSTYRVVSVLTVLHQDWLNGKEYKCKVSNKALAAPIEKTISKAKGQPREPQVCTLPPSRDELTKNQVSLSCAVKGFYPSDIAVEWESNGQPENNYKTTPPVLDSDGSFFLVSKLTVDKSRWQQGNVFSCSVMHEALHNHYTQKSLSLSPGK

SEQ ID NO: 118 - protein, 450 aa, artificial sequence
QVQLVQSGAEVKKPGASVKVSCKASGYTFTDYNIHWVRQAPGQGLEWMGYIYPYNGVSDYNQNFKSRVTMTTDTSTSTAYMELRSLRSDDTAVYYCARWDFGSGYYFDYWGQGTLVTVSSASTKGPSVFPLAPSSKSTSGGTAALGCLVKDYFPEPVTVSWNSGALTSGVHTFPAVLQSSGLYSLSSVVTVPSSSLGTQTYICNVNHKPSNTKVDKKVEPKSCDKTHTCPPCPAPEAAGGPSVFLFPPKPKDTLMISRTPEVTCVVVAVSHEDPEVKFNWYVDGVEVHNAKTKPREEQYNSTYRVVSVLTVLHQDWLNGKEYKCKVSNKALAAPIEKTISKAKGQPREPQVYTLPPCRDELTKNQVSLWCLVKGFYPSDIAVEWESNGQPENNYKTTPPVLDSDGSFFLYSKLTVDKSRWQQGNVFSCSVMHEALHNHYTQKSLSLSPGK

SEQ ID NO: 119 - protein, 673 aa, artificial sequence
QVQLVQSGAEVKKPGASVKVSCKASGYTFTDYNIHWVRQAPGQGLEWMGYIYPYNGVSDYNQNFKSRVTMTTDTSTSTAYMELRSLRSDDTAVYYCARWDFGSGYYFDYWGQGTLVTVSSASTKGPSVFPLAPSSKSTSGGTAALGCLVKDYFPEPVTVSWNSGALTSGVHTFPAVLQSSGLYSLSSVVTVPSSSLGTQTYICNVNHKPSNTKVDKKVEPKSCQVQLVQSGAEVKKPGASVKVSCKASGYTFTDYNIHWVRQAPGQGLEWMGYIYPYNGVSDYNQNFKSRVTMTTDTSTSTAYMELRSLRSDDTAVYYCARWDFGSGYYFDYWGQGTLVTVSSASTKGPSVFPLAPSSKSTSGGTAALGCLVKDYFPEPVTVSWNSGALTSGVHTFPAVLQSSGLYSLSSVVTVPSSSLGTQTYICNVNHKPSNTKVDKKVEPKSCDKTHTCPPCPAPEAAGGPSVFLFPPKPKDTLMISRTPEVTCVVVAVSHEDPEVKFNWYVDGVEVHNAKTKPREEQYNSTYRVVSVLTVLHQDWLNGKEYKCKVSNKALAAPIEKTISKAKGQPREPQVYTLPPCRDELTKNQVSLWCLVKGFYPSDIAVEWESNGQPENNYKTTPPVLDSDGSFFLYSKLTVDKSRWQQGNVFSCSVMHEALHNHYTQKSLSLSPGK

SEQ ID NO: 120 - protein, 720 aa, artificial sequence
MALPVTALLLPLALLLHAARPGSRKFNTTERVLQGLLRPLFKNTSVGPLYSGCRLTLLRPEKDGEATGVDVICTHRPDPTGPGLDREQLYLELSQLTHSITELGPYTLDNDSLFVNGFTHRSSVPTTSTGMVSEEPFTLNFTINNLRYMADMGQPGSLKFNITDNVMQHLLSPLFQRSSVGARYTGCRVIALRSVKNGAKTQVDILCTYLQPLSGPGLPIKQVFHELSQQTHGITRLGPYFLDKDSLYLNGYNEPGPDEPPTTPKPATTFLPPLSEATTAMGYHLKTLTLNFTISNLQYSPDMGNGSAAFNSTERVLKHLLRALFQKSSMGPFYLGCQLISLRPEKNGAATGVDTTCTYHTDPVGPGLDIQQLYWELSQLTHGVTQLGFYVLDRDSLFINGYAPQNLSIRGKYQIHFHIVNWNLGNPDPTSSEYIALLRDIQDKVTTLYKGSRLHDTFCYCLVTNLTMDSMLVTVKALFSSDLDPSLVEQVFLDKTLNASSHWLGSTYQLVDIHVTEMEPSVYQPTKPTSSSSTQHFYLNFTITNLPYSQDISQPSTTNYQRNKRNIEDALNQLFRNSSIKSCFSDCQVSTFRSVPNSHHTGVDSLCNFSPLARRVDRVAIYEEFLRMTRNGSQLQNFTLDRSSVLVDGYSPNRNEPLTGNSDLPFWAIILICLAVLLGLITCLICGFLATTRWRKKEEYSFRQQCPGYYRSHLDLEDLQ

SEQ ID NO: 121 - protein, 705 aa, artificial sequence
QVQLVQSGAEVKKPGASVKVSCKASGYTFTDYNIHWVRQAPGQGLEWMGYIYPYNGVSDYNQNFKSRVTMTTDTSTSTAYMELRSLRSDDTAVYYCARWDFGSGYYFDYWGQGTLVTVSSASTKGPSVFPLAPSSKSTSGGTAALGCLVKDYFPEPVTVSWNSGALTSGVHTFPAVLQSSGLYSLSSVVTVPSSSLGTQTYICNVNHKPSNTKVDKKVEPKSCEVQLVESGGGLVQPGGSLKLSCAASGFTFSTYAMNWVRQAPGKGLEWVGRIRSKYNNYATYYADSVKDRFTISRDDSKNTLYLQMNSLKTEDTAVYYCTRHGNFGNSYVSWFAYWGQGTTVTVSSGGGGSGGGGSGGGGSQAVVTQEPSLTVSPGGTVTLTCRSSTGAVTTSNYANWVQQKPGQAPRGLIGGTNKRAPGVPARFSGSLLGGKAALTLSGAQPEDEAEYFCALWYSNLWVFGGGTKLTVLGEPKSSDKTHTCPPCPAPEAAGGPSVFLFPPKPKDTLMISRTPEVTCVVVAVSHEDPEVKFNWYVDGVEVHNAKTKPREEQYNSTYRVVSVLTVLHQDWLNGKEYKCKVSNKALAAPIEKTISKAKGQPREPQVCTLPPSRDELTKNQVSLSCAVKGFYPSDIAVEWESNGQPENNYKTTPPVLDSDGSFFLVSKLTVDKSRWQQGNVFSCSVMHEALHNHYTQKSLSLSPGK

SEQ ID NO: 122 - protein, 443 aa, artificial sequence
QVQLVESGGGLVKPGGSLRLSCAASGFTFSNYYMSWVRQAPGKGLEWISYISGRGSTIFYADSVKGRITISRDNAKNSLFLQMNSLRAEDTAVYFCVKDRGGYSPYWGQGTLVTVSSASTKGPSVFPLAPCSRSTSESTAALGCLVKDYFPEPVTVSWNSGALTSGVHTFPAVLQSSGLYSLSSVVTVPSSSLGTKTYTCNVDHKPSNTKVDKRVESKYGPPCPPCPAPPVAGPSVFLFPPKPKDTLMISRTPEVTCVVVDVSQEDPEVQFNWYVDGVEVHNAKTKPREEQFNSTYRVVSVLTVLHQDWLNGKEYKCKVSNKGLPSSIEKTISKAKGQPREPQVYTLPPSQEEMTKNQVSLTCLVKGFYPSDIAVEWESNGQPENNYKTTPPVLDSDGSFFLYSRLTVDKSRWQEGNVFSCSVMHEALHNHYTQKSLSLSLGK

SEQ ID NO: 123 - protein, 450 aa, artificial sequence
EVQLVESGGGLVQPGRSLRLSCAASGFTFDDYSMHWVRQAPGKGLEWVSGISWNSGSIGYADSVKGRFTISRDNAKNSLYLQMNSLRAEDTALYYCAKYGSGYGKFYYYGMDVWGQGTTVTVSSASTKGPSVFPLAPCSRSTSESTAALGCLVKDYFPEPVTVSWNSGALTSGVHTFPAVLQSSGLYSLSSVVTVPSSSLGTKTYTCNVDHKPSNTKVDKRVESKYGPPCPPCPAPPVAGPSVFLFPPKPKDTLMISRTPEVTCVVVDVSQEDPEVQFNWYVDGVEVHNAKTKPREEQFNSTYRVVSVLTVLHQDWLNGKEYKCKVSNKGLPSSIEKTISKAKGQPREPQVYTLPPSQEEMTKNQVSLTCLVKGFYPSDIAVEWESNGQPENNYKTTPPVLDSDGSFFLYSRLTVDKSRWQEGNVFSCSVMHEALHNRFTQKSLSLSLGK

SEQ ID NO: 124 - protein, 215 aa, artificial sequence
DIQMTQSPSSLSASVGDRVTITCRASQSISTYLNWYQQKPGKAPKLLIYTASSLQSGVPSRFSGSGSGTDFTLTISSLQPEDFATYYCQQSYSTPPITFGQGTRLEIKRTVAAPSVFIFPPSDEQLKSGTASVVCLLNNFYPREAKVQWKVDNALQSGNSQESVTEQDSKDSTYSLSSTLTLSKADYEKHKVYACEVTHQGLSSPVTKSFNRGEC

SEQ ID NO: 125 - protein, 116 aa, artificial sequence
EVQLVESGGGLVQPGGSLRLSCAASGYSITNDYAWNWVRQAPGKGLEWVGYISYSGYTTYNPSLKSRFTISRDTSKNTLYLQMNSLRAEDTAVYYCARWTSGLDYWGQGTLVTVSS

SEQ ID NO: 126 - protein, 107 aa, artificial sequence
DIQMTQSPSSLSASVGDRVTITCKASDLIHNWLAWYQQKPGKAPKLLIYGATSLETGVPSRFSGSGSGTDFTLTISSLQPEDFATYYCQQYWTTPFTFGQGTKVEIK

SEQ ID NO: 127 - protein, 718 aa, artificial sequence
MALPVTALLLPLALLLHAARPGSRKFNTTERVLQGLLRPLFKNTSVGPLYSGCRLTLLRPEKDGEATGVDAICTHRPDPTGPGLDREQLYLELSQLTHSITELGPYTLDRDSLYVNGFTHRSSVPTTSTGVVSEEPFTLNFTINNLRYMADMGQPGSLKFNITDNVMQHLLSPLFQRSSLGARYTGCRVIALRSVKNGAETRVDLLCTYLQPLSGPGLPIKQVFHELSQQTHGITRLGPYSLDKDSLYLNGYNEPGPDEPPTTPKPATTFLPPLSEATTAMGYHLKTLTLNFTISNLQYSPDMGKGSATFNSTEGVLQHLLRPLFQKSSMGPFYLGCQLISLRPEKDGAATGVDTTCTYHPDPVGPGLDIQQLYWELSQLTHGVTQLGFYVLDRDSLFINGYAPQNLSIRGEYQINFHIVNWNLSNPDPTSSEYITLLRDIQDKVTTLYKGSQLHDTFRFCLVTNLTMDSVLVTVKALFSSNLDPSLVEQVFLDKTLNASFHWLGSTYQLVDIHVTEMESSVYQPTSSSSTQHFYLNFTITNLPYSQDKAQPGTTNYQRNKRNIEDALNQLFRNSSIKSYFSDCQVSTFRSVPNRHHTGVDSLCNFSPLARRVDRVAIYEEFLRMTRNGTQLQNFTLDRSSVLVDGYSPNRNEPLTGNSDLPFWAVILIGLAGLLGVITCLICGVLVTTRRRKKEGEYNVQQQCPGYYQSHLDLEDLQ

SEQ ID NO: 128 - protein, 720 aa, artificial sequence
MALPVTALLLPLALLLHAARPGSRKFNTTERVLQGLLRPLFKNTSVGPLYSGCRLTLLRPEKDGEATGVDVICTHRPDPTGPGLDREQLYLELSQLTHSITELGPYTLDNDSLFVNGFTHRSSVPTTSTGMVSEEPFTLNFTINNLRYMADMGQPGSLKFNITDNVMQHLLSPLFQRSSVGARYTGCRVIALRSVKNGAKTQVDILCTYLQPLSGPALPIKQVFHELSQQTHGITRLGPYFLDKDSLYLNGYNEPGPDEPPTTPKPATTFLPPLSEATTAMGYHLKTLTLNFTISNLQYSPDMGNGSAAFNSTERVLKHLLRALFQKSSMGPFYLGCQLISLRPEKNGAATGVDTTCTYHTDPVGPGLDIQQLYWELSQLTHGVTQLGFYVLDRDSLFINGYAPQNLSIRGKYQIHFHIVNWNFSNPDPTSSEYIALLRDIQDKVTTLYKGSQLHDTFRYCLVTNLTMDSMLVTVKALFSSDLDPSLVEQVFLDKTLNASSHWLGSTYQLVDIHVTEMEPSVYQPTKPTSSSSTQHFYLNFTITNLPYSQDISQPSTTNYQRNKRNIEDALNQLFRNSSIKSYFSDCQVSTFRSVPNSHHTGVDSLCNFSPLARRVDRVAIYEEFLRMTRNGSQLQNFTLDRSSVLVDGYSPNRNEPLTGNSDLPFWAIILICLAVLLGLITCLICGFLATTRWRKKEEYSFRQQCPGYYRSHLDLEDLQ